European Patent Application EP 4 261 231 A1, published October 18, 2023. Title: Bispecific antibody and application thereof. Applicant: QURE BIOTECHNOLOGY (SHANGHAI) CO., LTD. Application PCT/CN2021/094672. The sequence listing filed with the application follows.

SEQUENCE LISTING (19 sequences)

SEQ ID NO: 1 - protein, 114 aa, Artificial Sequence
  IL15
NWVNVISDLKKIEDLIQSMHIDATLYTESDVHPSCKVTAMKCFLLELQVISLESGDASIHDTVENLIILANNSLSSNGNVTESGCKECEELEEKNIKEFLQSFVHIVQMFINTS

SEQ ID NO: 2 - protein, 114 aa, Artificial Sequence
  IL-15(L52C)
NWVNVISDLKKIEDLIQSMHIDATLYTESDVHPSCKVTAMKCFLLELQVISCESGDASIHDTVENLIILANNSLSSNGNVTESGCKECEELEEKNIKEFLQSFVHIVQMFINTS

SEQ ID NO: 3 - protein, 178 aa, Artificial Sequence
  IL15Ra
ECDITCPPPMSVEHADIWVKSYSLYSRERYICNSGFKRKAGTSSLTECVLNKATNVAHWTTPSLKCIRDPALVHQRPAPPSTVTTAGVTPQPESLSPSGKEPAASSPSSNNTAATTAAIVPGSQLMPSKSPSTGTTEISSHESSHGTPSQTTAKNWELTASASHQPPGVYPQGHSDTT

SEQ ID NO: 4 - protein, 65 aa, Artificial Sequence
  IL15Ra Sushi 65">sp|Q13261|31-95
ITCPPPMSVEHADIWVKSYSLYSRERYICNSGFKRKAGTSSLTECVLNKATNVAHWTTPSLKCIR

SEQ ID NO: 5 - protein, 73 aa, Artificial Sequence
  IL15Ra Sushi 73
ITCPPPMSVEHADIWVKSYSLYSRERYICNSGFKRKAGTSSLTECVLNKATNVAHWTTPSLKCIRDPALVHQR

SEQ ID NO: 6 - protein, 77 aa, Artificial Sequence
  IL15Ra Sushi 77
ITCPPPMSVEHADIWVKSYSLYSRERYICNSGFKRKAGTSSLTECVLNKATNVAHWTTPSLKCIRDPALVHQRPAPP

SEQ ID NO: 7 - protein, 86 aa, Artificial Sequence
  IL15Ra Sushi 86
ITCPPPMSVEHADIWVKSYSLYSRERYICNSGFKRKAGTSSLTECVLNKATNVAHWTTPSLKCIRDPALVHQRPAPPSTVTTAGVT

SEQ ID NO: 8 - protein, 102 aa, Artificial Sequence
  IL15Ra Sushi 102
ITCPPPMSVEHADIWVKSYSLYSRERYICNSGFKRKAGTSSLTECVLNKATNVAHWTTPSLKCIRDPALVHQRPAPPSTVTTAGVTPQPESLSPSGKEPAAS

SEQ ID NO: 9 - protein, 65 aa, Artificial Sequence
  IL15Ra-sushi(S40C)
ITCPPPMSVEHADIWVKSYSLYSRERYICNSGFKRKAGTCSLTECVLNKATNVAHWTTPSLKCIR

SEQ ID NO: 10 - protein, 236 aa, Artificial Sequence
  anti Her2 VL-IL15
DIQMTQSPSSLSASVGDRVTITCRASQDVNTAVAWYQQKPGKAPKLLIYSASFLYSGVPSRFSGSRSGTDFTLTISSLQPEDFATYYCQQHYTTPPTFGQGTKVEIKGGGGSGGGGSGGGGSNWVNVISDLKKIEDLIQSMHIDATLYTESDVHPSCKVTAMKCFLLELQVISCESGDASIHDTVENLIILANNSLSSNGNVTESGCKECEELEEKNIKEFLQSFVHIVQMFINTS

SEQ ID NO: 11 - protein, 437 aa, Artificial Sequence
  anti Her2 VH-IL15Ra-Fc(Knob
EVQLVESGGGLVQPGGSLRLSCAASGFNIKDTYIHWVRQAPGKGLEWVARIYPTNGYTRYADSVKGRFTISADTSKNTAYLQMNSLRAEDTAVYYCSRWGGDGFYAMDYWGQGTLVTVSSGGGGSGGGGSGGGGSITCPPPMSVEHADIWVKSYSLYSRERYICNSGFKRKAGTCSLTECVLNKATNVAHWTTPSLKCIRGGGGSEPKSSDKTHTCPPCPAPELLGGPSVFLFPPKPKDTLMISRTPEVTCVVVDVSHEDPEVKFNWYVDGVEVHNAKTKPREEQYNSTYRVVSVLTVLHQDWLNGKEYKCKVSNKALPAPIEKTISKAKGQPREPQVYTLPPSRDELTKNQVSLWCLVKGFYPSDIAVEWESNGQPENNYKTTPPVLDSDGSFFLYSKLTVDKSRWQQGNVFSCSVMHEALHNHYTQKSLSLSPGK

SEQ ID NO: 12 - protein, 214 aa, Artificial Sequence
  anti Her2 VL-CL(Knob
DIQMTQSPSSLSASVGDRVTITCKASQDVSIGVAWYQQKPGKAPKLLIYSASYRYTGVPSRFSGSGSGTDFTLTISSLQPEDFATYYCQQYYIYPYTFGQGTKVEIKRTVAAPSVFIFPPSDEQLKSGTASVVCLLNNFYPREAKVQWKVDNALQSGNSQESVTEQDSKDSTYSLSSTLTLSKADYEKHKVYACEVTHQGLSSPVTKSFNRGEC

SEQ ID NO: 13 - protein, 449 aa, Artificial Sequence
  anti Her2 VH-CH1-CH2-CH3(Hole
EVQLVESGGGLVQPGGSLRLSCAASGFTFTDYTMDWVRQAPGKGLEWVADVNPNSGGSIYNQRFKGRFTLSVDRSKNTLYLQMNSLRAEDTAVYYCARNLGPSFYFDYWGQGTLVTVSSASTKGPSVFPLAPSSKSTSGGTAALGCLVKDYFPEPVTVSWNSGALTSGVHTFPAVLQSSGLYSLSSVVTVPSSSLGTQTYICNVNHKPSNTKVDKKVEPKSCDKTHTCPPCPAPELLGGPSVFLFPPKPKDTLMISRTPEVTCVVVDVSHEDPEVKFNWYVDGVEVHNAKTKPREEQYNSTYRVVSVLTVLHQDWLNGKEYKCKVSNKALPAPIEKTISKAKGQPREPQVYTLPPSRDELTKNQVSLSCAVKGFYPSDIAVEWESNGQPENNYKTTPPVLDSDGSFFLVSKLTVDKSRWQQGNVFSCSVMHEALHNRYTQKSLSLSPGK

SEQ ID NO: 14 - protein, 236 aa, Artificial Sequence
  anti CS1 VL-IL15
DIQMTQSPSSLSASVGDRVTITCKASQDVGIAVAWYQQKPGKVPKLLIYWASTRHTGVPDRFSGSGSGTDFTLTISSLQPEDVATYYCQQYSSYPYTFGQGTKVEIKGGGGSGGGGSGGGGSNWVNVISDLKKIEDLIQSMHIDATLYTESDVHPSCKVTAMKCFLLELQVISCESGDASIHDTVENLIILANNSLSSNGNVTESGCKECEELEEKNIKEFLQSFVHIVQMFINTS

SEQ ID NO: 15 - protein, 436 aa, Artificial Sequence
  anti CS1 VH-IL15Ra-FC(Knob
EVQLVESGGGLVQPGGSLRLSCAASGFDFSRYWMSWVRQAPGKGLEWIGEINPDSSTINYAPSLKDKFIISRDNAKNSLYLQMNSLRAEDTAVYYCARPDGNYWYFDVWGQGTLVTVSSGGGGSGGGGSGGGGSITCPPPMSVEHADIWVKSYSLYSRERYICNSGFKRKAGTCSLTECVLNKATNVAHWTTPSLKCIRGGGGSEPKSSDKTHTCPPCPAPELLGGPSVFLFPPKPKDTLMISRTPEVTCVVVDVSHEDPEVKFNWYVDGVEVHNAKTKPREEQYNSTYRVVSVLTVLHQDWLNGKEYKCKVSNKALPAPIEKTISKAKGQPREPQVYTLPPSRDELTKNQVSLWCLVKGFYPSDIAVEWESNGQPENNYKTTPPVLDSDGSFFLYSKLTVDKSRWQQGNVFSCSVMHEALHNHYTQKSLSLSPGK

SEQ ID NO: 16 - protein, 214 aa, Artificial Sequence
  anti CD38 VL-CL
EIVLTQSPATLSLSPGERATLSCRASQSVSSYLAWYQQKPGQAPRLLIYDASNRATGIPARFSGSGSGTDFTLTISSLEPEDFAVYYCQQRSNWPPTFGQGTKVEIKRTVAAPSVFIFPPSDEQLKSGTASVVCLLNNFYPREAKVQWKVDNALQSGNSQESVTEQDSKDSTYSLSSTLTLSKADYEKHKVYACEVTHQGLSSPVTKSFNRGEC

SEQ ID NO: 17 - protein, 452 aa, Artificial Sequence
  anti CD38 VH-CH1-CH2-CH3(Hole
EVQLLESGGGLVQPGGSLRLSCAVSGFTFNSFAMSWVRQAPGKGLEWVSAISGSGGGTYYADSVKGRFTISRDNSKNTLYLQMNSLRAEDTAVYFCAKDKILWFGEPVFDYWGQGTLVTVSSASTKGPSVFPLAPSSKSTSGGTAALGCLVKDYFPEPVTVSWNSGALTSGVHTFPAVLQSSGLYSLSSVVTVPSSSLGTQTYICNVNHKPSNTKVDKKVEPKSCDKTHTCPPCPAPELLGGPSVFLFPPKPKDTLMISRTPEVTCVVVDVSHEDPEVKFNWYVDGVEVHNAKTKPREEQYNSTYRVVSVLTVLHQDWLNGKEYKCKVSNKALPAPIEKTISKAKGQPREPQVYTLPPSRDELTKNQVSLSCAVKGFYPSDIAVEWESNGQPENNYKTTPPVLDSDGSFFLVSKLTVDKSRWQQGNVFSCSVMHEALHNRYTQKSLSLSPGK

SEQ ID NO: 18 - protein, 231 aa, Artificial Sequence
  Fc-KnobhIgG1)
EPKSCDKTHTCPPCPAPELLGGPSVFLFPPKPKDTLMISRTPEVTCVVVDVSHEDPEVKFNWYVDGVEVHNAKTKPREEQYNSTYRVVSVLTVLHQDWLNGKEYKCKVSNKALPAPIEKTISKAKGQPREPQVYTLPPSRDELTKNQVSLWCLVKGFYPSDIAVEWESNGQPENNYKTTPPVLDSDGSFFLYSKLTVDKSRWQQGNVFSCSVMHEALHNHYTQKSLSLSPG

SEQ ID NO: 19 - protein, 231 aa, Artificial Sequence
  Fc-Hole(hIgG1)
EPKSCDKTHTCPPCPAPELLGGPSVFLFPPKPKDTLMISRTPEVTCVVVDVSHEDPEVKFNWYVDGVEVHNAKTKPREEQYNSTYRVVSVLTVLHQDWLNGKEYKCKVSNKALPAPIEKTISKAKGQPREPQVYTLPPSRDELTKNQVSLSCAVKGFYPSDIAVEWESNGQPENNYKTTPPVLDSDGSFFLVSKLTVDKSRWQQGNVFSCSVMHEALHNHYTQKSLSLSPG